European Patent Application EP 4 357 458 A1, published April 24, 2024. Title: Inhibitors for Fra-1 and Fra-2 for use in the treatment of organ or tissue fibrosis. Applicant: Universitätsmedizin der Johannes Gutenberg-Universität Mainz. Application EP. The sequence listing filed with the application follows.

SEQUENCE LISTING (35 sequences)

SEQ ID NO: 1 - RNA, 21 nt, synthetic construct
  source 1..21: mol_type = other RNA
gctcaccgcagaagcagtatt

SEQ ID NO: 2 - RNA, 21 nt, synthetic construct
  source 1..21: mol_type = other RNA
tactgcttctgcggtgagctt

SEQ ID NO: 3 - RNA, 21 nt, synthetic construct
  source 1..21: mol_type = other RNA
gctcaccgcagaagcagtatt

SEQ ID NO: 4 - RNA, 21 nt, synthetic construct
  source 1..21: mol_type = other RNA
tactgcttctgcggtgagctt

SEQ ID NO: 5 - RNA, 21 nt, synthetic construct
  source 1..21: mol_type = other RNA
tcgaagtactcagcgtaagtt

SEQ ID NO: 6 - RNA, 22 nt, synthetic construct
  source 1..22: mol_type = other RNA
cttacgctgagtacttcgadtt

SEQ ID NO: 7 - DNA, 16 bp, unidentified
  source 1..16: mol_type = other DNA
acagccctcgcaccca

SEQ ID NO: 8 - DNA, 25 bp, unidentified
  source 1..25: mol_type = other DNA
caagatcattgcccctccagaacgc

SEQ ID NO: 9 - DNA, 20 bp, unidentified
  source 1..20: mol_type = other DNA
gccaccgatccagacagagt

SEQ ID NO: 10 - DNA, 19 bp, unidentified
  source 1..19: mol_type = other DNA
acgcatggccaagaagaca

SEQ ID NO: 11 - DNA, 21 bp, unidentified
  source 1..21: mol_type = other DNA
aagcatacctcgggtttccac

SEQ ID NO: 12 - DNA, 28 bp, unidentified
  source 1..28: mol_type = other DNA
agctgcatacacaatggcctaagggtcc

SEQ ID NO: 13 - DNA, 25 bp, unidentified
  source 1..25: mol_type = other DNA
cctgccaagtatgatgacatcaaga

SEQ ID NO: 14 - DNA, 25 bp, unidentified
  source 1..25: mol_type = other DNA
cctgccaagtatgatgacatcaaga

SEQ ID NO: 15 - DNA, 20 bp, unidentified
  source 1..20: mol_type = other DNA
tggtgaagcaggcggccgag

SEQ ID NO: 16 - DNA, 27 bp, unidentified
  source 1..27: mol_type = other DNA
tcctcttgttgctatcactgatagctt

SEQ ID NO: 17 - DNA, 23 bp, unidentified
  source 1..23: mol_type = other DNA
cgctggtataaggtggtctcgtt

SEQ ID NO: 18 - DNA, 27 bp, unidentified
  source 1..27: mol_type = other DNA
ttctgcaactcggacctggtcataagg

SEQ ID NO: 19 - DNA, 20 bp, unidentified
  source 1..20: mol_type = other DNA
agaggtcacccgcgtgctaa

SEQ ID NO: 20 - DNA, 22 bp, unidentified
  source 1..22: mol_type = other DNA
tcccgaatgtctgacgtattga

SEQ ID NO: 21 - DNA, 30 bp, unidentified
  source 1..30: mol_type = other DNA
accgcaacaacgccatctatgagaaaacca

SEQ ID NO: 22 - DNA, 19 bp, unidentified
  source 1..19: mol_type = other DNA
gagacgcgagcggaacaag

SEQ ID NO: 23 - DNA, 20 bp, unidentified
  source 1..20: mol_type = other DNA
cttccagcaccagctcaagg

SEQ ID NO: 24 - DNA, 19 bp, unidentified
  source 1..19: mol_type = other DNA
cactcccggcacttcaaac

SEQ ID NO: 25 - DNA, 20 bp, unidentified
  source 1..20: mol_type = other DNA
gagtctgatgactggtcccc

SEQ ID NO: 26 - DNA, 21 bp, unidentified
  source 1..21: mol_type = other DNA
aaggctatcctggtggaagaa

SEQ ID NO: 27 - DNA, 21 bp, unidentified
  source 1..21: mol_type = other DNA
agggaagggtcagtctgtgtt

SEQ ID NO: 28 - DNA, 22 bp, unidentified
  source 1..22: mol_type = other DNA
ctccaagccaaagtccttagag

SEQ ID NO: 29 - DNA, 22 bp, unidentified
  source 1..22: mol_type = other DNA
aggagctgtcattagggacatc

SEQ ID NO: 30 - DNA, 32 bp, unidentified
  source 1..32: mol_type = other DNA
ctatctccattctactactactaccagatcga

SEQ ID NO: 31 - DNA, 20 bp, unidentified
  source 1..20: mol_type = other DNA
cctgggcctcagcttctcat

SEQ ID NO: 32 - DNA, 23 bp, unidentified
  source 1..23: mol_type = other DNA
accagaggaaattttcaataggc

SEQ ID NO: 33 - DNA, 20 bp, unidentified
  source 1..20: mol_type = other DNA
tgatgcacttgcagaaaaca

SEQ ID NO: 34 - DNA, 21 bp, unidentified
  source 1..21: mol_type = other DNA
gctcttactgactggcatgag

SEQ ID NO: 35 - DNA, 20 bp, unidentified
  source 1..20: mol_type = other DNA
cgcagctctaggagcatgtg